European Patent Specification EP 3 911 959 B1, published July 3, 2024. Title: High speed sample workflow for LC-MS based HbA1c measurement. Applicant: Roche Diagnostics GmbH F. Hoffmann-La Roche AG. The sequence listing filed with the application follows.

SEQUENCE LISTING (1 sequence)

SEQ ID NO: 1 - protein, 16 aa, Homo sapiens
VHLTPEEKSAVTALWG